European Patent Application EP 4 516 309 A1, published March 5, 2025. Title: CRHR1 agonists for use in the treatment of social anxiety disorders. Applicant: Consejo Superior de Investigaciones Cientificas (CSIC). The sequence listing filed with the application follows.

SEQUENCE LISTING (8 sequences)

SEQ ID NO: 1 - protein, 40 aa, Homo sapiens
SEEPPISLDLTFHLLREVLEMARAEQLAQQAHSNRKLMEI

SEQ ID NO: 2 - DNA, 21 bp, synthetic construct
  source 1..21: mol_type = other DNA
gcccttgaatttcttgcagcc

SEQ ID NO: 3 - DNA, 21 bp, synthetic construct
  source 1..21: mol_type = other DNA
gcatgggtgaagaatacttcc

SEQ ID NO: 4 - DNA, 21 bp, synthetic construct
  source 1..21: mol_type = other DNA
ggaaactgatggagattatcg

SEQ ID NO: 5 - DNA, 23 bp, synthetic construct
  source 1..23: mol_type = other DNA
ccccgcagcccttgaatttcttg

SEQ ID NO: 6 - DNA, 21 bp, synthetic construct
  source 1..21: mol_type = other DNA
gggcgtggagttgggggacag

SEQ ID NO: 7 - DNA, 24 bp, synthetic construct
  source 1..24: mol_type = other DNA
gcaaattccatggcaccgtcaagg

SEQ ID NO: 8 - DNA, 20 bp, synthetic construct
  source 1..20: mol_type = other DNA
cgccagcatcgccccacttg